European Patent Specification EP 4 025 559 B1, published July 15, 2026. Title: ANTI-FIBROTIC COMPOUNDS AND USE THEREOF. Applicant: HADASIT MEDICAL RESEARCH SERVICES AND DEVELOPMENT LTD. RICHTER-DAYAN, Shulamit BREUER, Raphael SERTCHOOK, Rotem. The sequence listing filed with the application follows.

SEQUENCE LISTING (2 sequences)

SEQ ID NO: 1 - DNA, 67 bp, Artificial Sequence
  synthetic oligonucleotide
cgcgtccccgaatagacttgaacacaaattcaagagatttgtgttcaagtctattctttttggaaat

SEQ ID NO: 2 - DNA, 65 bp, Artificial Sequence
  Synthetic oligonucleotide
aggggcttatctgaacttgtgtttaagttctctaaacacaagttcagataagaaaaacctttagc